European Patent Specification EP 3 946 356 B1, published August 27, 2025. Title: Compound and method for the prevention of transmision of influenza virus. Applicant: F. Hoffmann-La Roche AG Shionogi & Co., Ltd. The sequence listing filed with the application follows.

SEQUENCE LISTING (5 sequences)

SEQ ID NO: 1 - DNA, 21 bp, Artificial Sequence
  Forward primer for real-time PCR
gaccratcctgtcacctctga

SEQ ID NO: 2 - DNA, 24 bp, Artificial Sequence
  Reverse primer for real-time PCR
agggcattytggacaaakcgtcta

SEQ ID NO: 3 - DNA, 24 bp, Artificial Sequence
  Probe for real-time PCR
tcgagtcctcgctcactgggcacg

SEQ ID NO: 4 - protein, 716 aa, Influenza A virus (A/WSN/1933(H1N1))
MEDFVRQCFNPMIVELAEKAMKEYGEDLKIETNKFAATCTHLEVCFMYSDFHFIDEQGESIVVELGDPNALLKHRFEIIEGRDRTIAWTVINSICNTTGAEKPKFLPDLYDYKKNRFIEIGVTRREVHIYYLEKANKIKSEKTHIHIFSFTGEEMATKADYTLDEESRARIKTRLFTIRQEMASRGLWDSFRQSERGEETIEERFEITGTMRKLADQSLPPNFSSLENFRAYVDGFEPNGYIEGKLSQMSKEVNARIEPFLKSTPRPLRLPDGPPCSQRSKFLLMDALKLSIEDPSHEGEGIPLYDAIKCMRTFFGWKEPNVVKPHEKGINPNYLLSWKQVLAELQDIENEEKIPRTKNMKKTSQLKWALGENMAPEKVDFDDCKDVGDLKQYDSDEPELRSLASWIQNEFNKACELTDSSWIELDEIGEDAAPIEHIASMRRNYFTAEVSHCRATEYIMKGVYINTALLNASCAAMDDFQLIPMISKCRTKEGRRKTNLYGFIIKGRSHLRNDTDVVNFVSMEFSLTDPRLEPHKWEKYCVLEVGDMLLRSAIGHVSRPMFLYVRTNGTSKIKMKWGMEMRRCLLQSLQQIESMIEAESSVKEKDMTKEFFENKSETWPVGESPKGVEEGSIGKVCRTLLAKSVFNSLYASPQLEGFSAESRKLLLIVQALRDNLEPGTFDLGGLYEAIEECLINDPWVLLNASWFNSFLTHALR

SEQ ID NO: 5 - protein, 7 aa, Artificial Sequence
  Sequence fraction of Influenza A virus (A/WSN/1933(H1N1))
FAATCTH